European Patent Specification EP 3 577 456 B9, published October 4, 2023. Title: Fluorescent fusion polypeptide capable of detecting phosphorylation of cellular membrane receptors by GRKs (G-protein receptor kinases) and/or Receptor tyrosine kinases (RTKs). Applicant: INNOVATIVE TECHNOLOGIES IN BIOLOGICAL SYSTEMS SL. Application EP17382049.9. The sequence listing filed with the application follows.

SEQUENCE LISTING (4 sequences)

SEQ ID NO: 1 - DNA, 1701 bp, Artificial Sequence
  phosphorylated receptor binding peptide from b-arrestin
atggacagctacctgctgatgtggggcctgctgaccttcatcatggtgcccggctgccaggccgagctgtgcgacgacgacccccctgagatcccccacgccaccttcaaagccatggcctacaaagaaggcaccatgctgaactgcgagtgcaagcggggcttccggcggatcaagagcggcagcctgtacatgctgtgcaccggcaacagcagccacagcagctgggacaaccagtgccagtgcaccagcagcgccacccggaacaccaccaaacaggtcacaccccagcccgaggaacagaaagagcgcaagaccaccgagatgcagagccccatgcagcccgtggaccaggcctctctgcccggccactgcagagagcccccaccttgggagaacgaggccaccgagcggatctaccacttcgtggtcggacagatggtgtactaccagtgcgtgcagggctaccgggccctgcacagaggacctgccgagagcgtgtgcaagatgacccacggcaagacccggtggacccagccccagctgatctgcaccggcgagatggaaaccagccagttccccggcgaggaaaagccccaggccagccctgagggcagacccgagagcgagacaagctgcctggtgacaaccaccgacttccagatccagaccgagatggccgccacaatggaaacctccatcttcaccaccgacctgcaggtggccgtggccggctgcgtgttcctgctgatctctgtgctgctcctgagcggcctgacctggcagcggagacagagaaagagcggccggaccatcgggatccaactagttgtcgaccagcagcagcagcagcagggaattctgcagtcgacggtaccaatggtgggtgaggatagcgagctgatcaccgagaacatgcacatgaaactgtacatggagggcaccgtgaacaaccaccacttcaagtgcacatccgagggcgaaggcaagccctacgagggcacccagaccatgaagatcaaggtggtcgagggcggccctctccccttcgccttcgacatcctggctaccagcttcatgtacggcagcaaagccttcatcaaccacacccagggcatccccgacttctttaagcagtccttccctgagggcttcacatgggagagaatcaccacatacgaagacgggggcgtgctgaccgctacccaggacaccagcctccagaacggctgcctcatctacaacgtcaagatcaacggggtgaacttcccatccaacggccctgtgatgcagaagaaaacactcggctgggaggccagcaccgagatgctgtaccccgctgacagcggcctgagaggccatggccagatggccctgaagctcgtgggcgggggctacctgcactgctccctcaagaccacatacagatccaagaaacccgctaagaacctcaagatgcccggcttccacttcgtggaccacagactggaaagaatcaaggaggccgacaaagagacctacgtcgagcagcacgagatggctgtggccaagtactgcgacctccctagcaaactggggcacagcagatctcgagtaggcggcggcggctatggccgtgaagacctggatgtgctgggcttgtccttccgcaaagacctgggcggcctcattgaatttggcggcggccggcttcggctgaag

SEQ ID NO: 2 - protein, 567 aa, Artificial Sequence
  phosphorylated receptor binding peptide from b-arrestin
MDSYLLMWGLLTFIMVPGCQAELCDDDPPEIPHATFKAMAYKEGTMLNCECKRGFRRIKSGSLYMLCTGNSSHSSWDNQCQCTSSATRNTTKQVTPQPEEQKERKTTEMQSPMQPVDQASLPGHCREPPPWENEATERIYHFVVGQMVYYQCVQGYRALHRGPAESVCKMTHGKTRWTQPQLICTGEMETSQFPGEEKPQASPEGRPESETSCLVTTTDFQIQTEMAATMETSIFTTDLQVAVAGCVFLLISVLLLSGLTWQRRQRKSGRTIGIQLVVDQQQQQQGILQSTVPMVGEDSELITENMHMKLYMEGTVNNHHFKCTSEGEGKPYEGTQTMKIKVVEGGPLPFAFDILATSFMYGSKAFINHTQGIPDFFKQSFPEGFTWERITTYEDGGVLTATQDTSLQNGCLIYNVKINGVNFPSNGPVMQKKTLGWEASTEMLYPADSGLRGHGQMALKLVGGGYLHCSLKTTYRSKKPAKNLKMPGFHFVDHRLERIKEADKETYVEQHEMAVAKYCDLPSKLGHSRSRVGGGGYGREDLDVLGLSFRKDLGGLIEFGGGRLRLK

SEQ ID NO: 3 - protein, 272 aa, Artificial Sequence
  extracellular domain of interleukin-2 receptor
MDSYLLMWGLLTFIMVPGCQAELCDDDPPEIPHATFKAMAYKEGTMLNCECKRGFRRIKSGSLYMLCTGNSSHSSWDNQCQCTSSATRNTTKQVTPQPEEQKERKTTEMQSPMQPVDQASLPGHCREPPPWENEATERIYHFVVGQMVYYQCVQGYRALHRGPAESVCKMTHGKTRWTQPQLICTGEMETSQFPGEEKPQASPEGRPESETSCLVTTTDFQIQTEMAATMETSIFTTDLQVAVAGCVFLLISVLLLSGLTWQRRQRKSGRTI

SEQ ID NO: 4 - protein, 31 aa, Artificial Sequence
  Chlatrin and beta-adaptin peptide from arrestin
YGREDLDVLGLSFRKDLGGLIEFGGGRLRLK